European Patent Specification EP 4 023 059 B1, published November 6, 2024. Title: NON-HUMAN ANIMALS CAPABLE OF DH-DH REARRANGEMENT AND USES THEREOF. Applicant: Regeneron Pharmaceuticals, Inc. MURPHY, Andrew J. MACDONALD, Lynn GUO, Chunguang MCWHIRTER, John VORONINA, Vera. The sequence listing filed with the application follows.

SEQUENCE LISTING (151 sequences)

SEQ ID NO: 1 - DNA, 22 bp, Artificial Sequence
  hIgHJ2
gaggctgtgctactggtacttc

SEQ ID NO: 2 - DNA, 21 bp, Artificial Sequence
  hIgHJ2
ccgtggcaccctggtcactgt

SEQ ID NO: 3 - DNA, 19 bp, Artificial Sequence
  hIgHJ2
tggtgcctggacagagaag

SEQ ID NO: 4 - DNA, 21 bp, Artificial Sequence
  VI741-42h1
tttttgtgcaccccttaatgg

SEQ ID NO: 5 - DNA, 22 bp, Artificial Sequence
  VI741-42h1
atgtggtattacgatttttgga

SEQ ID NO: 6 - DNA, 27 bp, Artificial Sequence
  VI741-42h1
ctctgtgacactgtgggtataataacc

SEQ ID NO: 7 - DNA, 24 bp, Artificial Sequence
  VI742h2
tgtcacagagtccatcaaaaacct

SEQ ID NO: 8 - DNA, 14 bp, Artificial Sequence
  VI742h2
caccaccccctctc

SEQ ID NO: 9 - DNA, 19 bp, Artificial Sequence
  VI742h2
cctgagaccctggcaagct

SEQ ID NO: 10 - DNA, 19 bp, Artificial Sequence
  Neo
ggtggagaggctattcggc

SEQ ID NO: 11 - DNA, 23 bp, Artificial Sequence
  Neo
tgggcacaacagacaatcggctg

SEQ ID NO: 12 - DNA, 17 bp, Artificial Sequence
  Neo
gaacacggcggcatcag

SEQ ID NO: 13 - DNA, 19 bp, Artificial Sequence
  Jxn DH2-2
atggcgcttgcagcgattc

SEQ ID NO: 14 - DNA, 28 bp, Artificial Sequence
  Jxn DH2-2
ccaatactaacgaggaaatgcaaaccca

SEQ ID NO: 15 - DNA, 21 bp, Artificial Sequence
  Jxn DH2-2
accctcactgttgtccttctg

SEQ ID NO: 16 - DNA, 23 bp, Artificial Sequence
  Jxn DH2-8
gcaaacgtccatctgaaggagaa

SEQ ID NO: 17 - DNA, 27 bp, Artificial Sequence
  Jxn DH2-8
caaataaacgatggcaggctacacccg

SEQ ID NO: 18 - DNA, 22 bp, Artificial Sequence
  Jxn DH2-8
gagttgccgaaccgacttattg

SEQ ID NO: 19 - DNA, 23 bp, Artificial Sequence
  Jxn DH2-15
gcaatggtaggttcatgtccatc

SEQ ID NO: 20 - DNA, 20 bp, Artificial Sequence
  Jxn DH2-15
accgccgctggtactccaat

SEQ ID NO: 21 - DNA, 19 bp, Artificial Sequence
  Jxn DH2-15
ccctggctgtctgggtttg

SEQ ID NO: 22 - DNA, 21 bp, Artificial Sequence
  hIgHJ6
cagcagagggttccatgagaa

SEQ ID NO: 23 - DNA, 22 bp, Artificial Sequence
  hIgHJ6
caggacagggccacggacagtc

SEQ ID NO: 24 - DNA, 20 bp, Artificial Sequence
  hIgHJ6
gccacccagagaccttctgt

SEQ ID NO: 25 - DNA, 20 bp, Artificial Sequence
  hIgH31
atcacactcatcccatcccc

SEQ ID NO: 26 - DNA, 29 bp, Artificial Sequence
  hIgH31
cccttccctaagtaccacagagtgggctc

SEQ ID NO: 27 - DNA, 20 bp, Artificial Sequence
  hIgH31
cacagggaagcaggaactgc

SEQ ID NO: 28 - DNA, 17 bp, Artificial Sequence
  mIgHp2
gccatgcaaggccaagc

SEQ ID NO: 29 - DNA, 24 bp, Artificial Sequence
  mIgHp2
ccaggaaaatgctgccagagcctg

SEQ ID NO: 30 - DNA, 24 bp, Artificial Sequence
  mIgHp2
agttcttgagccttagggtgctag

SEQ ID NO: 31 - DNA, 20 bp, Artificial Sequence
  mADAM6-1
ctgagcatggtgtcccatct

SEQ ID NO: 32 - DNA, 24 bp, Artificial Sequence
  mADAM6-1
tgcagataagtgtcatctgggcaa

SEQ ID NO: 33 - DNA, 24 bp, Artificial Sequence
  mADAM6-1
ccagagtactgtagtggctctaag

SEQ ID NO: 34 - DNA, 20 bp, Artificial Sequence
  hIgk5
ccccgtcctcctcctttttc

SEQ ID NO: 35 - DNA, 32 bp, Artificial Sequence
  hIgk5
tcatgtccattaacccatttaccttttgccca

SEQ ID NO: 36 - DNA, 19 bp, Artificial Sequence
  hIgk5
tgcaagtgctgccagcaag

SEQ ID NO: 37 - DNA, 23 bp, Artificial Sequence
  hIgK21
catttggctacatatcaaagccg

SEQ ID NO: 38 - DNA, 27 bp, Artificial Sequence
  hIgK21
cctgagccagggaacagcccactgata

SEQ ID NO: 39 - DNA, 20 bp, Artificial Sequence
  hIgK21
acatggctgaggcagacacc

SEQ ID NO: 40 - DNA, 20 bp, Artificial Sequence
  mIgKd2
gcaaacaaaaaccactggcc

SEQ ID NO: 41 - DNA, 37 bp, Artificial Sequence
  mIgKd2
ctgttcctctaaaactggactccacagtaaatggaaa

SEQ ID NO: 42 - DNA, 19 bp, Artificial Sequence
  mIgKd2
ggccacattccatgggttc

SEQ ID NO: 43 - DNA, 17 bp, Artificial Sequence
  hyg
tgcggccgatcttagcc

SEQ ID NO: 44 - DNA, 21 bp, Artificial Sequence
  hyg
acgagcgggttcggcccattc

SEQ ID NO: 45 - DNA, 18 bp, Artificial Sequence
  hyg
ttgaccgattccttgcgg

SEQ ID NO: 46 - DNA, 20 bp, Artificial Sequence
  hIgHD-J.1
tggcagctgttcaaccatgt

SEQ ID NO: 47 - DNA, 22 bp, Artificial Sequence
  hIgHD-J.1
atccactgtcccagacagcacc

SEQ ID NO: 48 - DNA, 20 bp, Artificial Sequence
  hIgHD-J.1
ggcggtttgtggagtttcct

SEQ ID NO: 49 - DNA, 20 bp, Artificial Sequence
  hIgHD-J.2
tgttgcctccctgcttctag

SEQ ID NO: 50 - DNA, 23 bp, Artificial Sequence
  hIgHD-J.2
cccagaccctcccttgttcctga

SEQ ID NO: 51 - DNA, 18 bp, Artificial Sequence
  hIgHD-J.2
ggcccacgcattgttcag

SEQ ID NO: 52 - DNA, 3263 bp, Artificial Sequence
  >p46458 (23-D3-3-12_delJ1-3 donor]
tacgtaccctggccaccgccacccgggcctctctgctgctgggaaaacaagtcagaaagcaagtggatgagaggtggcgtgacagacccagcttcagatctgctctaccggtataacttcgtataatgtatgctatacgaagttatatgcatggcctccgcgccgggttttggcgcctcccgcgggcgcccccctcctcacggcgagcgctgccacgtcagacgaagggcgcagcgagcgtcctgatccttccgcccggacgctcaggacagcggcccgctgctcataagactcggccttagaaccccagtatcagcagaaggacattttaggacgggacttgggtgactctagggcactggttttctttccagagagcggaacaggcgaggaaaagtagtcccttctcggcgattctgcggagggatctccgtggggcggtgaacgccgatgattatataaggacgcgccgggtgtggcacagctagttccgtcgcagccgggatttgggtcgcggttcttgtttgtggatcgctgtgatcgtcacttggtgagtagcgggctgctgggctggccggggctttcgtggccgccgggccgctcggtgggacggaagcgtgtggagagaccgccaagggctgtagtctgggtccgcgagcaaggttgccctgaactgggggttggggggagcgcagcaaaatggcggctgttcccgagtcttgaatggaagacgcttgtgaggcgggctgtgaggtcgttgaaacaaggtggggggcatggtgggcggcaagaacccaaggtcttgaggccttcgctaatgcgggaaagctcttattcgggtgagatgggctggggcaccatctggggaccctgacgtgaagtttgtcactgactggagaactcggtttgtcgtctgttgcgggggcggcagttatggcggtgccgttgggcagtgcacccgtacctttgggagcgcgcgccctcgtcgtgtcgtgacgtcacccgttctgttggcttataatgcagggtggggccacctgccggtaggtgtgcggtaggcttttctccgtcgcaggacgcagggttcgggcctagggtaggctctcctgaatcgacaggcgccggacctctggtgaggggagggataagtgaggcgtcagtttctttggtcggttttatgtacctatcttcttaagtagctgaagctccggttttgaactatgcgctcggggttggcgagtgtgttttgtgaagttttttaggcaccttttgaaatgtaatcatttgggtcaatatgtaattttcagtgttagactagtaaattgtccgctaaattctggccgtttttggcttttttgttagacgtcgagctagcctagattgggaacccgggtctctcgaattgttgacaattaatcatcggcatagtatatcggcatagtataatacgacaaggtgaggaactaaaccatccaccatgattgaacaagatggattgcacgcaggttctccggccgcttgggtggagaggctattcggctatgactgggcacaacagacaatcggctgctctgatgccgccgtgttccggctgtcagcgcaggggcgcccggttctttttgtcaagaccgacctgtccggtgccctgaatgaactgcaggacgaggcagcgcggctatcgtggctggccacgacgggcgttccttgcgcagctgtgctcgacgttgtcactgaagcgggaagggactggctgctattgggcgaagtgccggggcaggatctcctgtcatctcaccttgctcctgccgagaaagtatccatcatggctgatgcaatgcggcggctgcatacgcttgatccggctacctgcccattcgaccaccaagcgaaacatcgcatcgagcgagcacgtactcggatggaagccggtcttgtcgatcaggatgatctggacgaagagcatcaggggctcgcgccagccgaactgttcgccaggctcaaggcgcgcatgcccgacggcgaggatctcgtcgtgacccatggcgatgcctgcttgccgaatatcatggtggaaaatggccgcttttctggattcatcgactgtggccggctgggtgtggcggaccgctatcaggacatagcgttggctacccgtgatattgctgaagagcttggcggcgaatgggctgaccgcttcctcgtgctttacggtatcgccgctcccgattcgcagcgcatcgccttctatcgccttcttgacgagttcttctgaagatccgctgtaagtctgcagaaattgatgatctattaaacaataaagatgtccactaaaatggaagtttttcctgtcatactttgttaagaagggtgagaacagagtacctacattttgaatggaaggattggagctacgggggtgggggtggggtgggattagataaatgcctgctctttactgaaggctctttactattgctttatgataatgtttcatagttggatatcataatttaaacaagcaaaaccaaattaagggccagctcattcctcccactcatgatctatagatctatagatctctcgtgggatcattgtttttctcttgattcccactttgtggttctaagtactgtggtttccaaatgtgtcagtttcatagcctgaagaacgagatcagcagcctctgttccacatacacttcattctcagtattgttttgccaagttctaattccatcagacctcgacctgcagccggcgcgccataacttcgtataatgtatgctatacgaagttatgtcgacctcgagaatttacaaaagaaaaggaaaaacacacttggcagccttcagcactctaatgattcttaacagcagcaaattattggcacaagactccagagtgactggcagggttgagggctggggtctcccacgtgttttggggctaacagcggaagggagagcactggcaaaggtgctgggggcccctggacccgacccgccctggagaccgcagccacatcagcccccagccccacaggccccctaccagccgcagggtttttgtgcaccccttaatggggcctcccacaatgtggtattacgatttttggagtggttattatacccacagtgtcacagagtccatcaaaaaccaagatggctttccttctgcctcctttctctgggcccagcgtcctctgtcctggagctgggagataatgtccgggggctccttggtctgcgctgggccatgtacgta

SEQ ID NO: 53 - DNA, 23 bp, Artificial Sequence
  DNA recognition site
tcagaaagcaagtggatgagagg

SEQ ID NO: 54 - DNA, 42 bp, Artificial Sequence
  5' D7.27 gRNA
ucagaaagcaaguggaugagguuuuagagcuaugcuguuuug

SEQ ID NO: 55 - DNA, 23 bp, Artificial Sequence
  DNA recognition site
gctccaggacagaggacgctggg

SEQ ID NO: 56 - DNA, 42 bp, Artificial Sequence
  3' JH1-3 del gRNA
gcuccaggacagaggacgcuguuuuagagcuaugcuguuuug

SEQ ID NO: 57 - DNA, 19 bp, Artificial Sequence
  5' up detect D7-27
gtgaacaggtggaaccaac

SEQ ID NO: 58 - DNA, 21 bp, Artificial Sequence
  3' ub pro-200
ccagtgccctagagtcaccca

SEQ ID NO: 59 - DNA, 21 bp, Artificial Sequence
  5' neo detect
ctcccactcatgatctataga

SEQ ID NO: 60 - DNA, 20 bp, Artificial Sequence
  3' down detect JH1-3 del
gtcccagttcccaaagaaag

SEQ ID NO: 61 - DNA, 3263 bp, Artificial Sequence
  >p46459 (23-D3-3-12_delJ1-5 donor)
tacgtaccctggccaccgccacccgggcctctctgctgctgggaaaacaagtcagaaagcaagtggatgagaggtggcgtgacagacccagcttcagatctgctctaccggtataacttcgtataatgtatgctatacgaagttatatgcatggcctccgcgccgggttttggcgcctcccgcgggcgcccccctcctcacggcgagcgctgccacgtcagacgaagggcgcagcgagcgtcctgatccttccgcccggacgctcaggacagcggcccgctgctcataagactcggccttagaaccccagtatcagcagaaggacattttaggacgggacttgggtgactctagggcactggttttctttccagagagcggaacaggcgaggaaaagtagtcccttctcggcgattctgcggagggatctccgtggggcggtgaacgccgatgattatataaggacgcgccgggtgtggcacagctagttccgtcgcagccgggatttgggtcgcggttcttgtttgtggatcgctgtgatcgtcacttggtgagtagcgggctgctgggctggccggggctttcgtggccgccgggccgctcggtgggacggaagcgtgtggagagaccgccaagggctgtagtctgggtccgcgagcaaggttgccctgaactgggggttggggggagcgcagcaaaatggcggctgttcccgagtcttgaatggaagacgcttgtgaggcgggctgtgaggtcgttgaaacaaggtggggggcatggtgggcggcaagaacccaaggtcttgaggccttcgctaatgcgggaaagctcttattcgggtgagatgggctggggcaccatctggggaccctgacgtgaagtttgtcactgactggagaactcggtttgtcgtctgttgcgggggcggcagttatggcggtgccgttgggcagtgcacccgtacctttgggagcgcgcgccctcgtcgtgtcgtgacgtcacccgttctgttggcttataatgcagggtggggccacctgccggtaggtgtgcggtaggcttttctccgtcgcaggacgcagggttcgggcctagggtaggctctcctgaatcgacaggcgccggacctctggtgaggggagggataagtgaggcgtcagtttctttggtcggttttatgtacctatcttcttaagtagctgaagctccggttttgaactatgcgctcggggttggcgagtgtgttttgtgaagttttttaggcaccttttgaaatgtaatcatttgggtcaatatgtaattttcagtgttagactagtaaattgtccgctaaattctggccgtttttggcttttttgttagacgtcgagctagcctagattgggaacccgggtctctcgaattgttgacaattaatcatcggcatagtatatcggcatagtataatacgacaaggtgaggaactaaaccatccaccatgattgaacaagatggattgcacgcaggttctccggccgcttgggtggagaggctattcggctatgactgggcacaacagacaatcggctgctctgatgccgccgtgttccggctgtcagcgcaggggcgcccggttctttttgtcaagaccgacctgtccggtgccctgaatgaactgcaggacgaggcagcgcggctatcgtggctggccacgacgggcgttccttgcgcagctgtgctcgacgttgtcactgaagcgggaagggactggctgctattgggcgaagtgccggggcaggatctcctgtcatctcaccttgctcctgccgagaaagtatccatcatggctgatgcaatgcggcggctgcatacgcttgatccggctacctgcccattcgaccaccaagcgaaacatcgcatcgagcgagcacgtactcggatggaagccggtcttgtcgatcaggatgatctggacgaagagcatcaggggctcgcgccagccgaactgttcgccaggctcaaggcgcgcatgcccgacggcgaggatctcgtcgtgacccatggcgatgcctgcttgccgaatatcatggtggaaaatggccgcttttctggattcatcgactgtggccggctgggtgtggcggaccgctatcaggacatagcgttggctacccgtgatattgctgaagagcttggcggcgaatgggctgaccgcttcctcgtgctttacggtatcgccgctcccgattcgcagcgcatcgccttctatcgccttcttgacgagttcttctgaagatccgctgtaagtctgcagaaattgatgatctattaaacaataaagatgtccactaaaatggaagtttttcctgtcatactttgttaagaagggtgagaacagagtacctacattttgaatggaaggattggagctacgggggtgggggtggggtgggattagataaatgcctgctctttactgaaggctctttactattgctttatgataatgtttcatagttggatatcataatttaaacaagcaaaaccaaattaagggccagctcattcctcccactcatgatctatagatctatagatctctcgtgggatcattgtttttctcttgattcccactttgtggttctaagtactgtggtttccaaatgtgtcagtttcatagcctgaagaacgagatcagcagcctctgttccacatacacttcattctcagtattgttttgccaagttctaattccatcagacctcgacctgcagccggcgcgccataacttcgtataatgtatgctatacgaagttatgtcgacctcgagaatttacaaaagaaaaggaaaaacacacttggcagccttcagcactctaatgattcttaacagcagcaaattattggcacaagactccagagtgactggcagggttgagggctggggtctcccacgtgttttggggctaacagcggaagggagagcactggcaaaggtgctgggggcccctggacccgacccgccctggagaccgcagccacatcagcccccagccccacaggccccctaccagccgcagggtttttgtgcaccccttaatggggcctcccacaatgtggtattacgatttttggagtggttattatacccacagtgtcacagagtccatcaaaaacctcctcaccaccccctctctgagtccacttagggagactcagcttgccagggtctcagggtcagagtcttggaggcattttggaggtcaggaaagaaagcctacgta

SEQ ID NO: 62 - DNA, 23 bp, Artificial Sequence
  DNA recognition site
tcagaaagcaagtggatgagagg

SEQ ID NO: 63 - DNA, 42 bp, Artificial Sequence; identical to SEQ ID NO: 54
  5' D7.27 crRNA

SEQ ID NO: 64 - DNA, 23 bp, Artificial Sequence
  DNA recognition site
ttagggagactcagcttgccagg

SEQ ID NO: 65 - DNA, 42 bp, Artificial Sequence
  3' JH1-5 del crRNA
uuagggagacucagcuugccguuuuagagcuaugcuguuuug

SEQ ID NO: 66 - DNA, 19 bp, Artificial Sequence
  5' up detect D7-27
gtgaacaggtggaaccaac

SEQ ID NO: 67 - DNA, 21 bp, Artificial Sequence
  3' ub pro-200
ccagtgccctagagtcaccca

SEQ ID NO: 68 - DNA, 21 bp, Artificial Sequence
  5' neo detect
ctcccactcatgatctataga

SEQ ID NO: 69 - DNA, 19 bp, Artificial Sequence
  3' down detect JH1-5 del
acgcaatcatcacgacagc

SEQ ID NO: 70 - DNA, 3345 bp, Artificial Sequence
  >p51816 (12-D2-2-23 donor)
actagtagaagataagctccagacccccaagactgggacctgccttcctgccaccgcgccggcgatgcatccgggtaggggaggcgcttttcccaaggcagtctggagttgacaattaatcatcggcatagtatatcggcatagtataatacgacaaggtgaggaactaaaccatggagaaaaaaatcactggatataccaccgttgatatatcccaatggcatcgtaaagaacattttgaggcatttcagtcagttgctcaatgtacctataaccagaccgttcagctggatattacggcctttttaaagaccgtaaagaaaaataagcacaagttttatccggcctttattcacattcttgcccgcctgatgaatgctcatccggaattccgtatggcaatgaaagacggtgagctggtgatatgggatagtgttcacccttgttacaccgttttccatgagcaaactgaaacgttttcatcgctctggagtgaataccacgacgatttccggcagtttctacacatatattcgcaagatgtggcgtgttacggtgaaaacctggcctatttccctaaagggtttattgagaatatgtttttcgtctcagccaatccctgggtgagtttcaccagttttgatttaaacgtggccaatatggacaacttcttcgcccccgttttcaccatgggcaaatattatacgcaaggcgacaaggtgctgatgccgctggcgattcaggttcatcatgccgtttgtgatggcttccatgtcggcagaatgcttaatgaattacaacagtactgcgatgagtggcagggcggggcgtaaggatcctgccatttcattacctctttctccgcacccgacatagataaagcttatcgataccgtcgacctcgagggggggcccggtacccgccggcgcttgtagctccagacctccgtgcctcccccgaccacttactgttagataggcattgatctaggcacggggcgcgatgttgacacgggccagggagctgttccacaaagatcaaccccaaaccgggaccgcctggcactcgcgccgctgccacttccctctccatttgttcccagcacctctgtgctccctccctcctccctccttcaggggaacagcctgtgcagcccctccctgcaccccacaccctggggaggcccaaccctgcctccagccctttctcccccgctgctcttcctgcccatccagacaaccctggggtcccatccctgcagcctacaccctggtctccacccagacccctgtctctccctccagacacccctcccaggccaaccctgcacacgcaggccctccccttttctgctcccagagcctcaccctctaccctctgtgcctaccccctgcctcctcctgcccacaactcgagctcttcctctcctggggcccctgagccatggcactgaccgtgcactcccacccccacactgcccatgccctcaccttcctcctggacactctgaccccgctcccctcttggacccagccctggtatttccaggacaaaggctcacccaagtcttccccatgcaggcccttgccctcactgcccggttacacggcagcctcctgtgcacagaagcagggagctcagcccttccacaggcagaaggcactgaaagaaatcggcctccagcaccctgatgcacgtccgcctgtgtctctcactgcccgcacctgcagggaggctcggcactccctgtaaagacgagggatccaggcagcaacatcatgggagaatgcagggctcccagacagcccagccctctcgcaggcctctcctgggaagagacctgcagccaccactgaacagccacggagcccgctggatagtaactgagtcagtgaccgacctggagggcaggggagcagtgaaccggagcccagaccatagggacagagaccagccgctgacatcccgagcccctcactggcggccccagaacaccgcgtggaaacagaacagacccacattcccacctggaaaagggcagacactgctgagcccccagcaccagccctgagaaacaccaggcaacggcatcagagggggctcctgagaaagaaaggaggggaggtctccttcaccagcaagtacttcccttgaccaaaaacagggtccacgcaactcccccaggacaaaggaggagccccctgtacagcactgggctcagagtcctctcccacacaccctgagtttcagacaaaaaccccctggaaatcatagtatcagcaggagaactagccagagacagcaagaggggactcagtgactcccgcggggacaggaggattttgtgggggctcgtgtcactgtgaggatattgtagtagtaccagctgctatacccacagtgtgaaaacccacatcctgagagtgacacaaacccctgctgtaaacgcttccacttctggagctgaggggctggggggagcgtctgggaagtagggcctaggggtggccatcaatgcccaaaacgcaccagactcccccccagacatcaccccactggccagtgagcagagtaaacagaaaatgagaagcagctgggaagcttgcacaggccccaaggaaagagctttggcgggtgtgcaagaggggatgcgggcagagcctgagcagggccttttgctgtttctgctttcctgtgcagatagttccataaactggtgttcaagatcgatggctgggagtgagcccaggaggacagtgtgggaagggcacagggaaggagaagcagccgctatcctacactgtcatctttcaagagtttgccctgtgcccacaatgctgcatcatgggatgcttaacagctgatgtagacacagctaaagagagaatcagtgaaatggatttgcagcacagatctgaataaattctccagaatgtggagccacacagaagcaagcacaaggaaagtgcctgatgcaagggcaaagtacagtgtgtaccttcaggctgggcacagacactctgaaaagccttggcaggaactccctgcaacaaagcagagccctgcaggcaatgccagctccagagccctccctgagagcctcatgggcaaagatgtgcacaacaggtgtttctcatagccccaaactgagaatgaagcaaacagccatctgaaggaaaacaggcaaataaacgatggcaggttcatggcgcttgcagcgattcaacagctaaccaatactaacgaggaaatgcaaacccagacagccagaaggacaacagtgagggttacaggtgactctgtggttgagttcatgacaatgctgagtaattggagtaactagt

SEQ ID NO: 71 - DNA, 2484 bp, Artificial Sequence
  >p53419 (12-D2-8-23 donor)
actagtcccagtcctctcacaggcctctcctgggaagagacctgaagacgcccagtcgccggcgatgcatccgggtaggggaggcgcttttcccaaggcagtctggagttgacaattaatcatcggcatagtatatcggcatagtataatacgacaaggtgaggaactaaaccatggagaaaaaaatcactggatataccaccgttgatatatcccaatggcatcgtaaagaacattttgaggcatttcagtcagttgctcaatgtacctataaccagaccgttcagctggatattacggcctttttaaagaccgtaaagaaaaataagcacaagttttatccggcctttattcacattcttgcccgcctgatgaatgctcatccggaattccgtatggcaatgaaagacggtgagctggtgatatgggatagtgttcacccttgttacaccgttttccatgagcaaactgaaacgttttcatcgctctggagtgaataccacgacgatttccggcagtttctacacatatattcgcaagatgtggcgtgttacggtgaaaacctggcctatttccctaaagggtttattgagaatatgtttttcgtctcagccaatccctgggtgagtttcaccagttttgatttaaacgtggccaatatggacaacttcttcgcccccgttttcaccatgggcaaatattatacgcaaggcgacaaggtgctgatgccgctggcgattcaggttcatcatgccgtttgtgatggcttccatgtcggcagaatgcttaatgaattacaacagtactgcgatgagtggcagggcggggcgtaaggatcctgccatttcattacctctttctccgcacccgacatagataaagcttatcgataccgtcgacctcgagggggggcccggtacccgccggcgcaacggagtctaacaccaaacctccctggaggccgatgggcgagcaaaatccgacacgtaactacaagtagggcctgatctagtaacggagtcattgccagacctggaggcaggggagcagtgagcccgagcccacaccatagggccagagggcacagcaactgacatcccaagccactcactggtggtcccacaacaccccatggaaagaggacagacccacagtcccacctggaccagggcagagactgctgagacccagcaccagaaccaaccaagaaacaccaggcaacagcatcagagggggctctggcagaacagaggaggggaggtctccttcaccagcaggcgcttcccttgaccgaagacaggatccatgcaactcccccaggacaaaggaggagccccttgttcagcactgggctcagagtcctctccaagacacccagagtttcagacaaaaaccccctggaatgcacagtctcagcaggagagccagccagagccagcaagatggggctcagtgacacccgcagggacaggaggattttgtgggggctcgtgtcactgtgaggatattgtactaatggtgtatgctatacccacagtgtgaaaacccacatcctgagagtgacacaaacccctactgcaaacgcattccacttctggggctgaggggctgggggagcgtctgggaaatagggctcaggggtgtccatcaatgcccaaaacgcaccagactcccctccatacatcacacccaccagccagcgagcagagtaaacagaaaatgagaagcaagctggggaagcttgcacaggccccaaggaaagagctttggcgggtgtgtaagaggggatgcgggcagagcctgagcagggccttttgctgtttctgctttcctgtgcagagagttccataaactggtgttcgagatcaatggctgggagtgagcccaggaggacagcgtgggaagagcacagggaaggaggagcagccgctatcctacactgtcatctttcaaaagtttcccttgtgcccacattgctgcatcatgggatgcttaagagctgatgtagacacagctaaagagagaatcagtgagatggatttgcagcacagatctgaataaattctccagaatgtggagcagcacagaagcaagcacacagaaagtgcctgatgcaaggacaaagttcagtgggcaccttcaggcattgctgctgggcacagacattctgaaaagccctggcaggaactccctgtgacaaagcagaaccctcaggcaatgccagccccagagccctccctgagagcctcatgggcaaagatgtgcacaacaggtgtttctcatagccccaaactgagagcaaagcaaacgtccatctgaaggagaacaggcaaataaacgatggcaggctacacccgtgcatccaataagtcggttcggcaactcaacttcatgaaatgcaaacccagacagccacaagcacaaaagtacagggttataagcgactctggttgagttcatgacaatgctgagtaattgactagt

SEQ ID NO: 72 - DNA, 2321 bp, Artificial Sequence
  >p51818 (12-D2-15-23 donor)
actagtgagaccagccgctgacatcccgagctcctcaatggtggccccataacacacgccggcgatgcatccgggtaggggaggcgcttttcccaaggcagtctggagttgacaattaatcatcggcatagtatatcggcatagtataatacgacaaggtgaggaactaaaccatggagaaaaaaatcactggatataccaccgttgatatatcccaatggcatcgtaaagaacattttgaggcatttcagtcagttgctcaatgtacctataaccagaccgttcagctggatattacggcctttttaaagaccgtaaagaaaaataagcacaagttttatccggcctttattcacattcttgcccgcctgatgaatgctcatccggaattccgtatggcaatgaaagacggtgagctggtgatatgggatagtgttcacccttgttacaccgttttccatgagcaaactgaaacgttttcatcgctctggagtgaataccacgacgatttccggcagtttctacacatatattcgcaagatgtggcgtgttacggtgaaaacctggcctatttccctaaagggtttattgagaatatgtttttcgtctcagccaatccctgggtgagtttcaccagttttgatttaaacgtggccaatatggacaacttcttcgcccccgttttcaccatgggcaaatattatacgcaaggcgacaaggtgctgatgccgctggcgattcaggttcatcatgccgtttgtgatggcttccatgtcggcagaatgcttaatgaattacaacagtactgcgatgagtggcagggcggggcgtaaggatcctgccatttcattacctctttctccgcacccgacatagataaagcttatcgataccgtcgacctcgagggggggcccggtacccgccggcgcctaggaaacataacacacccacagccccacctggaacagatagatgcaccaatatctcccagtaagctcaagctcgcggggcagagactgctgagcccccagcaccagccccaagaaacaccaggcaacagtatcagagggggctcccgagaaagagaggaggggagatctccttcaccatcaaatgcttcccttgaccaaaaacagggtccacgcaactcccccaggacaaaggaggagccccctatacagcactgggctcagagtcctctctgagacaccctgagtttcagacaacaacccgctggaatgcacagtctcagcaggagaacagaccaaagccagcaaaagggacctcggtgacaccagtagggacaggaggattttgtgggggctcgtgtcactgtgaggatattgtagtggtggtagctgctactcccacagtgtgaaaacccacatcctgagagtgacacaaacccctactgcaaacacccccactcctggggctgaggggctaggggagcgtctgggaagtagggtccaggggtgtctatcaatgtccaaaatgcaccagactccccgccaaacaccaccccaccagccagcgagcagggtaaacagaaaatgagaggctctgggaagcttgcacaggccccaaggaaagagctttggcgggtgtgcaagaggggatgcaggcagagcctgagcagggccttttgctgtttctgctttcctgtgcagagagttccataaactggtgttcaagatcagtggctgggaatgagcccaggagggcagtctgtgggaagagcacagggaaggaggagcagccgctatcctacactgtcatctttcaaaagtttgccttgtgaccacactattgcatcatgggatgcttaagagctgatgtagacacagctaaagagagaatcagtgagatgaatttgcagcatagatctgaataaactctccagaatgtggagcagtacagaagcaaacacacagaaagtgcctgatgcaaggacaaagttcagtgggcaccttcaggcattgctgctgggcacagacactctgaaaagccctggcaggatctccctgcgacaaagcagaaccctcaggcaatgccagccccagagccctccctgagagcgtcatggggaaagatgtgcagaacagctgattatcatagactcaaactgagaacagagcaaacgtccatctgaagaacagtcaaataagcaatggtaggttcatgtccatctcatcggtcagtaaaaataccgccgctggtactccaatgcaaacccagacagccaggggacaacagtagagggctacaggcggctttgcggttgagttcatgacaatgctgagtaattggagtaactagt

SEQ ID NO: 73 - DNA, 40 bp, Artificial Sequence
  1 P51816(D2-2)
tgttagataggcattgatctaggcacggggcgcgatgttg

SEQ ID NO: 74 - DNA, 40 bp, Artificial Sequence
  2 P51816(D2-2)
gcgcttgcagcgattcaacagctaaccaatactaacgagg

SEQ ID NO: 75 - DNA, 40 bp, Artificial Sequence
  10 P53419(D2-8)
cgagcaaaatccgacacgtaactacaagtagggcctgatc

SEQ ID NO: 76 - DNA, 40 bp, Artificial Sequence
  16 P53419(D2-8)
ctacacccgtgcatccaataagtcggttcggcaactcaac

SEQ ID NO: 77 - DNA, 40 bp, Artificial Sequence
  8 P51818(D2-15)
atagatgcaccaatatctcccagtaagctcaagctcgcgg

SEQ ID NO: 78 - DNA, 40 bp, Artificial Sequence
  18 P51818(D2-15)
tccatctcatcggtcagtaaaaataccgccgctggtactc

SEQ ID NO: 79 - DNA, 20 bp, Artificial Sequence
  5' hIgHD HU2(h268)
gcagtaaccctcaggaagca

SEQ ID NO: 80 - DNA, 31 bp, Artificial Sequence
  3' hIgHD HU2 AgeI(h269)
cttccaccggtacagccacaccaaggtcatc

SEQ ID NO: 81 - DNA, 31 bp, Artificial Sequence
  5' hIgHD HD2 XhoI(h271)
cttccctcgaggaacactgtcagctcccaca

SEQ ID NO: 82 - DNA, 19 bp, Artificial Sequence
  3' hIgHD HD2(h272)
agatcctccatgcgtgctg

SEQ ID NO: 83 - DNA, 20 bp, Artificial Sequence
  5' hIgHD HU2 detect(h270)
tctcctctcgtcgcctctac

SEQ ID NO: 84 - DNA, 21 bp, Artificial Sequence
  3' ub pro-200
ccagtgccctagagtcaccca

SEQ ID NO: 85 - DNA, 21 bp, Artificial Sequence
  5' neo detect
ctcccactcatgatctataga

SEQ ID NO: 86 - DNA, 20 bp, Artificial Sequence
  3' hIgHD HD2 detect(h273)
gggtgcttgggtcctgttag

SEQ ID NO: 87 - DNA, 23 bp, Artificial Sequence
  5' D2-2 Cas9 DNA target
aggtctggagctacaagcggtgg

SEQ ID NO: 88 - DNA, 42 bp, Artificial Sequence
  5' D2-2 gRNA
aggucuggagcuacaagcggguuuuagagcuaugcuguuuug

SEQ ID NO: 89 - DNA, 23 bp, Artificial Sequence
  3' D2-2 Cas9 DNA target
aggacaacagtgagggttacagg

SEQ ID NO: 90 - DNA, 42 bp, Artificial Sequence
  3' D2-2 gRNA
aggacaacagugaggguuacguuuuagagcuaugcuguuuug

SEQ ID NO: 91 - DNA, 19 bp, Artificial Sequence
  5' up detect D2-2(h274)
gtcaaaggtggaggcagtg

SEQ ID NO: 92 - DNA, 21 bp, Artificial Sequence
  3' cm up detect
tccagctgaacggtctggtta

SEQ ID NO: 93 - DNA, 19 bp, Artificial Sequence
  D2-2seqF2
agcgattcaacagctaacc

SEQ ID NO: 94 - DNA, 20 bp, Artificial Sequence
  3' down detect D2-2(h275)
ccagtagaagtaacgaccac

SEQ ID NO: 95 - DNA, 80 bp, Artificial Sequence
  JO-1
ctccagacccccaagactgggacctgccttcctgccaccgcttgtagctccagacctccgtgcctcccccgaccacttac

SEQ ID NO: 96 - DNA, 19 bp, Artificial Sequence
  5' up detect D2-2(h274)
gtcaaaggtggaggcagtg

SEQ ID NO: 97 - DNA, 19 bp, Artificial Sequence
  D2-2seqR1
cccgtgcctagatcaatgc

SEQ ID NO: 98 - DNA, 19 bp, Artificial Sequence
  D2-2seqF1
aggcattgatctaggcacg

SEQ ID NO: 99 - DNA, 19 bp, Artificial Sequence
  D2-2seqR2
ctgttgaatcgctgcaagc

SEQ ID NO: 100 - DNA, 23 bp, Artificial Sequence
  5' D2-8 Cas9 DNA target
acctgaagacgcccagtcaacgg

SEQ ID NO: 101 - DNA, 42 bp, Artificial Sequence
  5' D2-8 crRNA
accugaagacgcccagucaaguuuuagagcuaugcuguuuug

SEQ ID NO: 102 - DNA, 23 bp, Artificial Sequence
  3' D2-8 Cas9 DNA target
gccacaagcacaaaagtacaggg

SEQ ID NO: 103 - DNA, 42 bp, Artificial Sequence
  3' D2-8 crRNA
gccacaagcacaaaaguacaguuuuagagcuaugcuguuuug

SEQ ID NO: 104 - DNA, 19 bp, Artificial Sequence
  5' up detect D2-8(h276)
gccttacccaagtctttcc

SEQ ID NO: 105 - DNA, 21 bp, Artificial Sequence
  3' cm up detect
tccagctgaacggtctggtta

SEQ ID NO: 106 - DNA, 19 bp, Artificial Sequence
  D2-8seqF2
tccaataagtcggttcggc

SEQ ID NO: 107 - DNA, 19 bp, Artificial Sequence
  3' down detect D2-8(h277)
gcagaagtaaccaccactg

SEQ ID NO: 108 - DNA, 80 bp, Artificial Sequence
  JO-2
tcacaggcctctcctgggaagagacctgaagacgcccagtcaacggagtctaacaccaaacctccctggaggccgatggg

SEQ ID NO: 109 - DNA, 19 bp, Artificial Sequence
  5' up detect D2-8(h276)
gccttacccaagtctttcc

SEQ ID NO: 110 - DNA, 20 bp, Artificial Sequence
  D2-8seqR1
gccctacttgtagttacgtg

SEQ ID NO: 111 - DNA, 19 bp, Artificial Sequence
  D2-8seqF1
gcaaaatccgacacgtaac

SEQ ID NO: 112 - DNA, 20 bp, Artificial Sequence
  D2-8seqR2
cgaaccgacttattggatgc

SEQ ID NO: 113 - DNA, 23 bp, Artificial Sequence
  5' D2-8 Cas9 DNA target
ggtggccccataacacacctagg

SEQ ID NO: 114 - DNA, 42 bp, Artificial Sequence
  5' D2-8 crRNA
gguggccccauaacacaccuguuuuagagcuaugcuguuuug

SEQ ID NO: 115 - DNA, 23 bp, Artificial Sequence
  3' D2-8 Cas9 DNA target
ggacaacagtagagggctacagg

SEQ ID NO: 116 - DNA, 42 bp, Artificial Sequence
  3' D2-8 crRNA
ggacaacaguagagggcuacguuuuagagcuaugcuguuuug

SEQ ID NO: 117 - DNA, 20 bp, Artificial Sequence
  5' up detect D2-15(h278)
gcactccctctaaagacaag

SEQ ID NO: 118 - DNA, 21 bp, Artificial Sequence
  3' cm up detect
tccagctgaacggtctggtta

SEQ ID NO: 119 - DNA, 19 bp, Artificial Sequence
  D2-15seqF2
gtaaaaataccgccgctgg

SEQ ID NO: 120 - DNA, 19 bp, Artificial Sequence
  3' down detect D2-15(h279)
gcattttcctgttcttgcg

SEQ ID NO: 121 - DNA, 80 bp, Artificial Sequence
  JO-3
gctgacatcccgagctcctcaatggtggccccataacacacctaggaaacataacacacccacagccccacctggaacag

SEQ ID NO: 122 - DNA, 20 bp, Artificial Sequence
  5' up detect D2-15(h278)*
gcactccctctaaagacaag

SEQ ID NO: 123 - DNA, 20 bp, Artificial Sequence
  D2-15seqR1
ctgggagatattggtgcatc

SEQ ID NO: 124 - DNA, 19 bp, Artificial Sequence
  D2-15seqF1
tgcaccaatatctcccagt

SEQ ID NO: 125 - DNA, 20 bp, Artificial Sequence
  D2-15seqR2
cggcggtatttttactgacc

SEQ ID NO: 126 - DNA, 21 bp, Artificial Sequence
  23D3.312-1
tttttgtgcaccccttaatgg

SEQ ID NO: 127 - DNA, 22 bp, Artificial Sequence
  23D3.312-1
atgtggtattacgatttttgga

SEQ ID NO: 128 - DNA, 26 bp, Artificial Sequence
  23D3.312-1
tctgtgacactgtgggtataataacc

SEQ ID NO: 129 - DNA, 22 bp, Artificial Sequence
  23D3.312-2
cccacagtgtcacagagtccat

SEQ ID NO: 130 - DNA, 24 bp, Artificial Sequence
  23D3.312-2
caagatggctttccttctgcctcc

SEQ ID NO: 131 - DNA, 19 bp, Artificial Sequence
  23D3.312-2
tcccagctccaggacagag

SEQ ID NO: 132 - DNA, 24 bp, Artificial Sequence
  23D3.312-3
tgtcacagagtccatcaaaaacct

SEQ ID NO: 133 - DNA, 14 bp, Artificial Sequence
  23D3.312-3
caccaccccctctc

SEQ ID NO: 134 - DNA, 19 bp, Artificial Sequence
  23D3.312-3
cctgagaccctggcaagct

SEQ ID NO: 135 - DNA, 19 bp, Artificial Sequence
  Jxn DH2-2
atggcgcttgcagcgattc

SEQ ID NO: 136 - DNA, 28 bp, Artificial Sequence
  Jxn DH2-2
ccaatactaacgaggaaatgcaaaccca

SEQ ID NO: 137 - DNA, 21 bp, Artificial Sequence
  Jxn DH2-2
accctcactgttgtccttctg

SEQ ID NO: 138 - DNA, 23 bp, Artificial Sequence
  Jxn DH2-8
gcaaacgtccatctgaaggagaa

SEQ ID NO: 139 - DNA, 27 bp, Artificial Sequence
  Jxn DH2-8
caaataaacgatggcaggctacacccg

SEQ ID NO: 140 - DNA, 22 bp, Artificial Sequence
  Jxn DH2-8
gagttgccgaaccgacttattg

SEQ ID NO: 141 - DNA, 23 bp, Artificial Sequence
  Jxn DH2-15
gcaatggtaggttcatgtccatc

SEQ ID NO: 142 - DNA, 20 bp, Artificial Sequence
  Jxn DH2-15
accgccgctggtactccaat

SEQ ID NO: 143 - DNA, 19 bp, Artificial Sequence
  Jxn DH2-15
ccctggctgtctgggtttg

SEQ ID NO: 144 - DNA, 7 bp, Artificial Sequence
  Artificial
cacagtg

SEQ ID NO: 145 - DNA, 9 bp, Artificial Sequence
  Artificial
acaaaaacc

SEQ ID NO: 146 - DNA, 29 bp, Artificial Sequence
  Template switching oligo
agcagtggtatcaacgcagagtacatggg

SEQ ID NO: 147 - DNA, 54 bp, Artificial Sequence
  1st round PCR primers IgM Constant
acactctttccctacacgacgctcttccgatctgggaagacatttgggaaggac

SEQ ID NO: 148 - DNA, 57 bp, Artificial Sequence
  1st round PCR primers PE2-PIIA
gtgactggagttcagacgtgtgctcttccgatctaagcagtggtatcaacgcagagt

SEQ ID NO: 149 - DNA, 68 bp, Artificial Sequence
  2nd round PCR Primers
  misc_feature (30)..(35): n is a, c, g, or t
aatgatacggcgaccaccgagatctacacnnnnnnacactctttccctacacgacgctcttccgatct

SEQ ID NO: 150 - DNA, 64 bp, Artificial Sequence
  2nd round PCR Primers
  misc_feature (25)..(30): n is a, c, g, or t
caagcagaagacggcatacgagatnnnnnngtgactggagttcagacgtgtgctcttccgatct

SEQ ID NO: 151 - DNA, 39 bp, Artificial Sequence
  23-mer RSS from VH1-69
cacagtgtgaaaacccacatcctgagagtgacacaaacc